European Patent Application EP 4 406 970 A1, published July 31, 2024. Title: Monoclonal antibody targeting TIGIT. Applicant: SHANGHAI CELGEN BIO-PHARMACEUTICAL CO., LTD. The sequence listing filed with the application follows.

SEQUENCE LISTING (143 sequences)

SEQ ID NO: 1 - DNA, 17 bp, Artificial
  Heavy chain primer rHa-1
aggaactgcaggtgtcc

SEQ ID NO: 2 - DNA, 20 bp, Artificial
  Heavy chain primer rHa-2
cagctacaggtgtccactcc

SEQ ID NO: 3 - DNA, 19 bp, Artificial
  Heavy chain primer rHa-3
tggcagcarcagctacagg

SEQ ID NO: 4 - DNA, 19 bp, Artificial
  Heavy chain primer rHa-4
ctgcctggtgacattccca

SEQ ID NO: 5 - DNA, 17 bp, Artificial
  Heavy chain primer rHa-5
ccaagctgtgtcctgtc

SEQ ID NO: 6 - DNA, 20 bp, Artificial
  Heavy chain primer rHa-6
ttttaaaaggtgtccagkgt

SEQ ID NO: 7 - DNA, 23 bp, Artificial
  Heavy chain primer rHa-7
cctgtcagtaactrcaggtgtcc

SEQ ID NO: 8 - DNA, 20 bp, Artificial
  Heavy chain primerrHa-8
ttttaaaaggggtccagtgt

SEQ ID NO: 9 - DNA, 19 bp, Artificial
  Heavy chain primer rHa-9
cgttcctggtatcctgtct

SEQ ID NO: 10 - DNA, 21 bp, Artificial
  Heavy chain primer rHa-10
atgaagttgtggytraactgg

SEQ ID NO: 11 - DNA, 18 bp, Artificial
  Heavy chain primer rHa-11
tgttggggctkaagtggg

SEQ ID NO: 12 - DNA, 23 bp, Artificial
  Heavy chain primer rHa-12
agaaggtgtgcacaccgctggac

SEQ ID NO: 13 - DNA, 31 bp, Artificial
  Heavy chain primer rHb-1
gggaattcgaggtgcagctgcaggagtctgg

SEQ ID NO: 14 - DNA, 22 bp, Artificial
  Heavy chain primer rHb-2
gctcagggaartagcccttgac

SEQ ID NO: 15 - DNA, 24 bp, Artificial
  Light chain primer rKb-1
rgtgcagattttcagcttcctgct

SEQ ID NO: 16 - DNA, 24 bp, Artificial
  Light chain primer rKb-2
tggacatgagggcycctgctcagt

SEQ ID NO: 17 - DNA, 24 bp, Artificial
  Light chain primer rKb-3
ctstggttgtctggtgttgaygga

SEQ ID NO: 18 - DNA, 22 bp, Artificial
  Light chain primer rKb-4
gttgctgctgctgtggcttaca

SEQ ID NO: 19 - DNA, 17 bp, Artificial
  Light chain primer rKb-5
gtatctggtacctgtgg

SEQ ID NO: 20 - DNA, 22 bp, Artificial
  Light chain primer rKb-6
tgcctgttaggctgttggtgct

SEQ ID NO: 21 - DNA, 25 bp, Artificial
  Light chain primer rKb-7
gctcagttccttggtctcctgttgc

SEQ ID NO: 22 - DNA, 27 bp, Artificial
  Light chain primer rKb-8
cagttcctgtttctgttartgctctgg

SEQ ID NO: 23 - DNA, 26 bp, Artificial
  Light chain primer rKb-9
tgctctggttatatggtgctgatggg

SEQ ID NO: 24 - DNA, 21 bp, Artificial
  Light chain primer rKb-10
actgaggcacctccagatgtt

SEQ ID NO: 25 - DNA, 24 bp, Artificial
  Light chain primer rKc-1
gayattgtgmtsacmcarwctmca

SEQ ID NO: 26 - DNA, 19 bp, Artificial
  Light chain primer rKc-2
tgggaagatggatacagtt

SEQ ID NO: 27 - protein, 119 aa, Artificial
  7103-01 VH Full-length sequence
QVQLQQPGAELVKPGASVKLSCKASGYTFISYNIYWVKQRPGQGLEWIGGVNPSNGNTNFNENFKSKATLTVDKSSSTAYMQLSSLTSDDSAVYFCTRGNYYGYEFAYWGQGTLVTVSA

SEQ ID NO: 28 - protein, 5 aa, Artificial
  7103-01 VH CDR1
SYNIY

SEQ ID NO: 29 - protein, 17 aa, Artificial
  7103-01 VH CDR2
GVNPSNGNTNFNENFKS

SEQ ID NO: 30 - protein, 10 aa, Artificial
  7103-01 VH CDR3
GNYYGYEFAY

SEQ ID NO: 31 - protein, 107 aa, Artificial
  7103-01 VL Full-length sequence
DIVMTQSHKFMSTSVGDRVSITCKASQHVSTAVAWYQQKPGQSPKLLIYSPSYRYTGVPDRFTGSGSGTDFTFTISSVQAEDLAVYYCQQHYSTPWTFGGGTKLEIK

SEQ ID NO: 32 - protein, 11 aa, Artificial
  7103-01 VL CDR1
KASQHVSTAVA

SEQ ID NO: 33 - protein, 7 aa, Artificial
  7103-01 VL CDR2
SPSYRYT

SEQ ID NO: 34 - protein, 9 aa, Artificial
  7103-01 VL CDR3
QQHYSTPWT

SEQ ID NO: 35 - protein, 119 aa, Artificial
  7103-02 VH Full-length sequence
EVQLQQSGPELVKPGASVKMSCKASGYTITSYVMHWVKQKPGQGLEWIGYINPYNDGTKYNEKFKGKATLTSDKSSSTAYMELSSLTSEDSAVYYCARWNPYYYAMDYWGQGTSVTVSS

SEQ ID NO: 36 - protein, 5 aa, Artificial
  7103-02 VH CDR1
SYVMH

SEQ ID NO: 37 - protein, 17 aa, Artificial
  7103-02 VH CDR2
YINPYNDGTKYNEKFKG

SEQ ID NO: 38 - protein, 10 aa, Artificial
  7103-02 VH CDR3
WNPYYYAMDY

SEQ ID NO: 39 - protein, 106 aa, Artificial
  7103-02 VL Full-length sequence
EVVLTQSPAITAASLGQKVTITCSANSSARYVHWYQQKSGTSPKPWIYEISKLASGVPARFSGSGSGTSYSLTISSMGAEDAAIYYCQQWNYPLITFGAGTKLEIK

SEQ ID NO: 40 - protein, 10 aa, Artificial
  7103-02 VL CDR1
SANSSARYVH

SEQ ID NO: 41 - protein, 7 aa, Artificial
  7103-02 VL CDR2
EISKLAS

SEQ ID NO: 42 - protein, 9 aa, Artificial
  7103-02 VL CDR3
QQWNYPLIT

SEQ ID NO: 43 - protein, 119 aa, Artificial
  7103-03 VH Full-length sequence
EVQLQQSGPELVKPGASVKISCKTSGYTFTEYTMHWVKQSHGKSLEWIGGINPNNGGTSYNQKFKGKATLTVDKSSSTAYMELRSLTSEDSAVYYCARGAYYRYDFDYWGQGTTLTVSS

SEQ ID NO: 44 - protein, 5 aa, Artificial
  7103-03 VH CDR1
EYTMH

SEQ ID NO: 45 - protein, 17 aa, Artificial
  7103-03 VH CDR2
GINPNNGGTSYNQKFKG

SEQ ID NO: 46 - protein, 10 aa, Artificial
  7103-03 VH CDR3
GAYYRYDFDY

SEQ ID NO: 47 - protein, 107 aa, Artificial
  7103-03 VL Full-length sequence
DIVMTQSHKFMSTSVGDRVSITCKASQDVRTAVVWYQQKPGQSPKLLIYSASYRYTGVPDRFTGSGSGTDFTFTISSVQAEDLAVYYCQQHYSTPWTFGGGTKLEIK

SEQ ID NO: 48 - protein, 11 aa, Artificial
  7103-03 VL CDR1
KASQDVRTAVV

SEQ ID NO: 49 - protein, 7 aa, Artificial
  7103-03 VL CDR2
SASYRYT

SEQ ID NO: 50 - protein, 9 aa, Artificial
  7103-03 VL CDR3
QQHYSTPWT

SEQ ID NO: 51 - protein, 118 aa, Artificial
  7103-04 VH Full-length sequence
VQLQESGAELVKPGASVKLSCRASGYTFTDYFVYWVKQRPGQGLEWIGGINPSNGGATFNEKFKNKATLTVDTSSSTAYMQLSSLTSEDSAIYYCTRGNFYGYEFAYWGQGTLVTVSA

SEQ ID NO: 52 - protein, 5 aa, Artificial
  7103-04 VH CDR1
DYFVY

SEQ ID NO: 53 - protein, 17 aa, Artificial
  7103-04 VH CDR2
GINPSNGGATFNEKFKN

SEQ ID NO: 54 - protein, 10 aa, Artificial
  7103-04 VH CDR3
GNFYGYEFAY

SEQ ID NO: 55 - protein, 107 aa, Artificial
  7103-04 VL Full-length sequence
DIVMTQSHKFISTSVGDRVSITCKASQHVSTAVVWYQQKPGQSPKLLIYSPSYRYTGVPDRFTGSGSGTDFTFTISSVQAEDLAVYYCQQHYITPWTFGGGTKLEIK

SEQ ID NO: 56 - protein, 11 aa, Artificial
  7103-04 VL CDR1
KASQHVSTAVV

SEQ ID NO: 57 - protein, 7 aa, Artificial
  7103-04 VL CDR2
SPSYRYT

SEQ ID NO: 58 - protein, 9 aa, Artificial
  7103-04 VL CDR3
QQHYITPWT

SEQ ID NO: 59 - protein, 119 aa, Artificial
  7103-05 VH Full-length sequence
EVQLQQSGPALVKPGASVKISCKTSEYTFTEYTMYWVKQSHGKSLEWIGGINPNNGGTRYNQKFKGKATLTVDKSSSTAYMELRSLTSEDSAVYYCARGGHYDYGFAYWGQGTLVTVSA

SEQ ID NO: 60 - protein, 5 aa, Artificial
  7103-05 VH CDR1
EYTMY

SEQ ID NO: 61 - protein, 17 aa, Artificial
  7103-05 VH CDR2
GINPNNGGTRYNQKFKG

SEQ ID NO: 62 - protein, 10 aa, Artificial
  7103-05 VH CDR3
GGHYDYGFAY

SEQ ID NO: 63 - protein, 107 aa, Artificial
  7103-05 VL Full-length sequence
DIVMTQSHKFMSTSVGDRVSITCKASQDVKTAVAWYQQKPGQSPKVLIYSPSYRYTGVPDRFTGSGSGTDFTFTISSVQAEDLAVYYCQQHYSTPWTFGGGTKLKSK

SEQ ID NO: 64 - protein, 11 aa, Artificial
  7103-05 VL CDR1
KASQDVKTAVA

SEQ ID NO: 65 - protein, 7 aa, Artificial
  7103-05 VL CDR2
SPSYRYT

SEQ ID NO: 66 - protein, 9 aa, Artificial
  7103-05 VL CDR3
QQHYSTPWT

SEQ ID NO: 67 - protein, 119 aa, Artificial
  7103-06 VH Full-length sequence
EEQLVESGGGLVKPGGTLKLSCAASGFTFSTYAMSWVRQSPEKRLEWVAEISSGGSYTYYSDTVTGRFTISRDNAKNTLYLEMSSLRSEDTAMYYCARKTLDYYALDYWGHGTSVTVSS

SEQ ID NO: 68 - protein, 5 aa, Artificial
  7103-06 VH CDR1
TYAMS

SEQ ID NO: 69 - protein, 17 aa, Artificial
  7103-06 VH CDR2
EISSGGSYTYYSDTVTG

SEQ ID NO: 70 - protein, 10 aa, Artificial
  7103-06 VH CDR3
KTLDYYALDY

SEQ ID NO: 71 - protein, 107 aa, Artificial
  7103-06 VL Full-length sequence
DVQITQSPSYLAASPGETITINCRANKTISKYLAWYQEKPGKTNKLLIYSGSRLQSGIPSKFSGSGYGTDFTLTISSLEPEDFAMYYCQQHNEYPWTFGGGTKLEIK

SEQ ID NO: 72 - protein, 11 aa, Artificial
  7103-06 VL CDR1
RANKTISKYLA

SEQ ID NO: 73 - protein, 7 aa, Artificial
  7103-06 VL CDR2
SGSRLQS

SEQ ID NO: 74 - protein, 9 aa, Artificial
  7103-06 VL CDR3
QQHNEYPWT

SEQ ID NO: 75 - protein, 119 aa, Artificial
  7103-07 VH Full-length sequence
EVQVVESGGGLVKPGGTLKLSCAASGFTFSTYAMSWVRQSPEQRLEWVAEISSGGSHTFYSDTVTGRFTISRDNAQNTLYLEMNSLRSEDTAMYYCARKTLDYYALDYWGQGTSVTVSS

SEQ ID NO: 76 - protein, 5 aa, Artificial
  7103-07 VH CDR1
TYAMS

SEQ ID NO: 77 - protein, 17 aa, Artificial
  7103-07 VH CDR2
EISSGGSHTFYSDTVTG

SEQ ID NO: 78 - protein, 10 aa, Artificial
  7103-07 VH CDR3
KTLDYYALDY

SEQ ID NO: 79 - protein, 107 aa, Artificial
  7103-07 VL Full-length sequence
DVQITQSPSYLAASPGETITINCRASKSISKYLAWYQEKPGKTNKLLIYSGSRLQSGIPSKFSGSGYGTDFTLTISSLEPEDFAMYYCQQHNEYPWTFGGGTKVEIK

SEQ ID NO: 80 - protein, 11 aa, Artificial
  7103-07 VL CDR1
RASKSISKYLA

SEQ ID NO: 81 - protein, 7 aa, Artificial
  7103-07 VL CDR2
SGSRLQS

SEQ ID NO: 82 - protein, 9 aa, Artificial
  7103-07 VL CDR3
QQHNEYPWT

SEQ ID NO: 83 - protein, 116 aa, Artificial
  7103-08 VH Full-length sequence
EVQLQESGPELVKPGASVKISCKASGYSFTGYYMLWVKQSHVKSLEWIGRINPYNGATTYNQNFKDKASLTVNKSSSTAYMELHSLTSEDSAVYYCARWFGDFDFWGQGTTLTVSS

SEQ ID NO: 84 - protein, 5 aa, Artificial
  7103-08 VH CDR1
GYYML

SEQ ID NO: 85 - protein, 17 aa, Artificial
  7103-08 VH CDR2
RINPYNGATTYNQNFKD

SEQ ID NO: 86 - protein, 7 aa, Artificial
  7103-08 VH CDR3
WFGDFDF

SEQ ID NO: 87 - protein, 107 aa, Artificial
  7103-08 VL Full-length sequence
DIQMTQSPSSLSASLGERVSLTCRASQEISGYLSWLQQKPDGTIKRLIYATSTLDSGVPKRFSGSRSGSDYSLTISSLESEDFADYYCLQYASYPFTFGSGTKLEIK

SEQ ID NO: 88 - protein, 11 aa, Artificial
  7103-08 VL CDR1
RASQEISGYLS

SEQ ID NO: 89 - protein, 7 aa, Artificial
  7103-08 VL CDR2
ATSTLDS

SEQ ID NO: 90 - protein, 9 aa, Artificial
  7103-08 VL CDR3
LQYASYPFT

SEQ ID NO: 91 - DNA, 40 bp, Artificial
  Primer 7103-01-L-F
gcttcccaggcgccagatgcgacattgtgatgacmcagtc

SEQ ID NO: 92 - DNA, 40 bp, Artificial
  Primer 7103-01-L-R
atggagcggccacagtacgtttkatttccarcttkgtscc

SEQ ID NO: 93 - DNA, 40 bp, Artificial
  Primer 7103-02-L-F
gcttcccaggcgccagatgcgaaawtgtgctcacccagtc

SEQ ID NO: 94 - DNA, 40 bp, Artificial
  Primer 7103-02-L-R
atggagcggccacagtacgtttcagctccagcttggtccc

SEQ ID NO: 95 - DNA, 40 bp, Artificial; identical to SEQ ID NO: 91
  Primer 7103-03-L-F

SEQ ID NO: 96 - DNA, 40 bp, Artificial; identical to SEQ ID NO: 92
  Primer 7103-03-L-R

SEQ ID NO: 97 - DNA, 40 bp, Artificial; identical to SEQ ID NO: 91
  Primer 7103-04-L-F

SEQ ID NO: 98 - DNA, 40 bp, Artificial; identical to SEQ ID NO: 92
  Primer 7103-04-L-R

SEQ ID NO: 99 - DNA, 40 bp, Artificial; identical to SEQ ID NO: 91
  Primer 7103-05-L-F

SEQ ID NO: 100 - DNA, 40 bp, Artificial
  Primer 7103-05-L-F2
gcttcccaggcgccagatgcgacattgtgatgacacagtc

SEQ ID NO: 101 - DNA, 40 bp, Artificial; identical to SEQ ID NO: 92
  Primer 7103-05-L-R

SEQ ID NO: 102 - DNA, 40 bp, Artificial
  Primer 7103-06-L-F
gcttcccaggcgccagatgcgatgtccagataacccagtc

SEQ ID NO: 103 - DNA, 40 bp, Artificial; identical to SEQ ID NO: 92
  Primer 7103-06-L-R

SEQ ID NO: 104 - DNA, 40 bp, Artificial; identical to SEQ ID NO: 102
  Primer 7103-07-L-F

SEQ ID NO: 105 - DNA, 40 bp, Artificial; identical to SEQ ID NO: 92
  Primer 7103-07-L-R

SEQ ID NO: 106 - DNA, 40 bp, Artificial
  Primer 7103-08-L-F
gcttcccaggcgccagatgcgacatccagatgachcagtc

SEQ ID NO: 107 - DNA, 40 bp, Artificial; identical to SEQ ID NO: 92
  Primer 7103-08-L-R

SEQ ID NO: 108 - DNA, 37 bp, Artificial
  Primer 7103-01-H-F
taaaaggtgtccagtgtcaggtccaactgcagcagcc

SEQ ID NO: 109 - DNA, 37 bp, Artificial
  Primer 7103-01-H-R
ggcccctttgttgatgctgcagagacagtgaccagag

SEQ ID NO: 110 - DNA, 37 bp, Artificial
  Primer 7103-02-H-F
taaaaggtgtccagtgtsaggtycagctgcarcagtc

SEQ ID NO: 111 - DNA, 37 bp, Artificial
  Primer 7103-02-H-R
ggcccctttgttgatgctgaggagacggtgactgagg

SEQ ID NO: 112 - DNA, 37 bp, Artificial; identical to SEQ ID NO: 110
  Primer 7103-03-H-F

SEQ ID NO: 113 - DNA, 37 bp, Artificial
  Primer 7103-03-H-R
ggcccctttgttgatgctgaggagactgtgagagtgg

SEQ ID NO: 114 - DNA, 37 bp, Artificial; identical to SEQ ID NO: 110
  Primer 7103-04-H-F

SEQ ID NO: 115 - DNA, 37 bp, Artificial; identical to SEQ ID NO: 109
  Primer 7103-04-H-R

SEQ ID NO: 116 - DNA, 37 bp, Artificial; identical to SEQ ID NO: 110
  Primer 7103-05-H-F

SEQ ID NO: 117 - DNA, 37 bp, Artificial; identical to SEQ ID NO: 109
  Primer 7103-05-H-R

SEQ ID NO: 118 - DNA, 37 bp, Artificial
  Primer 7103-06-H-F
taaaaggtgtccagtgtgawgtgcagctggtggagtc

SEQ ID NO: 119 - DNA, 37 bp, Artificial; identical to SEQ ID NO: 111
  Primer 7103-06-H-R

SEQ ID NO: 120 - DNA, 37 bp, Artificial; identical to SEQ ID NO: 118
  Primer 7103-07-H-F

SEQ ID NO: 121 - DNA, 37 bp, Artificial; identical to SEQ ID NO: 111
  Primer 7103-07-H-R

SEQ ID NO: 122 - DNA, 37 bp, Artificial; identical to SEQ ID NO: 110
  Primer 7103-08-H-F

SEQ ID NO: 123 - DNA, 37 bp, Artificial; identical to SEQ ID NO: 113
  Primer 7103-08-H-R

SEQ ID NO: 124 - protein, 119 aa, Artificial
  7103-01 huVH1 Full-length sequence
QVQLVQSGAEVKKPGASVKLSCKASGYTFISYNIYWVRQAPGQGLEWIGGVNPSNGNTNFNENFKSRATLTVDKSSSTAYMELSRLRSDDTAVYFCTRGNYYGYEFAYWGQGTTVTVSS

SEQ ID NO: 125 - protein, 119 aa, Artificial
  7103-01 huVH2 Full-length sequence
QVQLVQSGAEVKKPGASVKVSCKASGYTFISYNIYWVRQAPGQGLEWIGGVNPSNGNTNFNENFKSRVTLTVDKSISTAYMELSRLRSDDTAVYYCTRGNYYGYEFAYWGQGTTVTVSS

SEQ ID NO: 126 - protein, 119 aa, Artificial
  7103-01 huVH3 Full-length sequence
QVQLVQSGAEVKKPGASVKVSCKASGYTFISYNIYWVRQAPGQGLEWIGGVNPSNGNTNFNENFKGRVTLTVDTSISTAYMELSRLRSDDTAVYYCTRGNYYGYEFAYWGQGTTVTVSS

SEQ ID NO: 127 - protein, 119 aa, Artificial
  7103-01 huVH4 Full-length sequence
QVQLVQSGAEVKKPGASVKVSCKASGYTFISYNIYWVRQAPGQGLEWMGGVNPSNGNTNFNENFQGRVTMTVDTSISTAYMELSRLRSDDTAVYYCTRGNYYGYEFAYWGQGTTVTVSS

SEQ ID NO: 128 - protein, 17 aa, Artificial
  7103-01 huVH4 CDR2
GVNPSNGNTNFNENFQG

SEQ ID NO: 129 - protein, 107 aa, Artificial
  7103-01 huVL1 Full-length sequence
DIQMTQSPSSMSASVGDRVTITCKASQHVSTAVAWYQQKPGKAPKLLIYSPSYRYTGVPSRFSGSGSGTDFTFTISSVQPEDIATYYCQQHYSTPWTFGGGTKLEIK

SEQ ID NO: 130 - protein, 107 aa, Artificial
  7103-01 huVL2 Full-length sequence
DIQMTQSPSSLSASVGDRVTITCKASQHVSTAVAWYQQKPGKAPKLLIYSPSYRYTGVPSRFSGSGSGTDFTFTISSLQPEDIATYYCQQHYSTPWTFGGGTKLEIK

SEQ ID NO: 131 - protein, 119 aa, Artificial
  7103-07 huVH1 Full-length sequence
EVQVVESGGGLVKPGGSLRLSCAASGFTFSTYAMSWVRQAPGKGLEWVAEISSGGSHTFYSDTVTGRFTISRDNAKNTLYLQMNSLRAEDTAVYYCARKTLDYYALDYWGQGTTVTVSS

SEQ ID NO: 132 - protein, 119 aa, Artificial
  7103-07 huVH2 Full-length sequence
EVQVVESGGGLVKPGGSLRLSCAASGFTFSTYAMSWVRQAPGKGLEWVAEISSGGSHTFYADTVKGRFTISRDNAKNTLYLQMNSLRAEDTAVYYCARKTLDYYALDYWGQGTTVTVSS

SEQ ID NO: 133 - protein, 17 aa, Artificial
  7103-07 huVH2 or huVH5 CDR2
EISSGGSHTFYADTVKG

SEQ ID NO: 134 - protein, 119 aa, Artificial
  7103-07 huVH3 Full-length sequence
EVQLVESGGGLVKPGGSLRLSCAASGFTFSTYAMSWVRQAPGKGLEWVAEISSGGSHTFYADTVTGRFTISRDNAKNTLYLQMNSLRAEDTAVYYCARKTLDYYALDYWGQGTTVTVSS

SEQ ID NO: 135 - protein, 119 aa, Artificial
  7103-07 huVH4 Full-length sequence
EVQVVESGGGLVKPGGSLRLSCAASGFTFSTYAMSWVRQAPEQRLEWVAEISSGGSHTFYSDTVTGRFTISRDNAKNTLYLQMNSLRAEDTAVYYCARKTLDYYALDYWGQGTTVTVSS

SEQ ID NO: 136 - protein, 119 aa, Artificial
  7103-07 huVH5 Full-length sequence
EVQVVESGGGLVKPGGSLRLSCAASGFTFSTYAMSWVRQAPEQRLEWVAEISSGGSHTFYADTVKGRFTISRDNAKNTLYLQMNSLRAEDTAVYYCARKTLDYYALDYWGQGTTVTVSS

SEQ ID NO: 137 - protein, 107 aa, Artificial
  7103-07 huVL1 Full-length sequence
DVQITQSPSYLSASVGDRVTINCRASKSISKYLAWYQQKPGKAPKLLIYSGSRLQSGIPSRFSGSGYGTDFTLTISSLQPEDFATYYCQQHNEYPWTFGGGTKLEIK

SEQ ID NO: 138 - protein, 107 aa, Artificial
  7103-07 huVL2 Full-length sequence
DVQITQSPSSVSASVGDRVTINCRASKSISKYLAWYQQKPGKAPKLLIYSGSRLQSGVPSRFSGSGSGTDFTLTISSLQPEDFATYYCQQHNEYPWTFGGGTKLEIK

SEQ ID NO: 139 - protein, 107 aa, Artificial
  7103-07 huVL3 Full-length sequence
DIQMTQSPSSVSASVGDRVTITCRASKSISKYLAWYQQKPGKAPKLLIYSGSRLQSGVPSRFSGSGSGTDFTLTISSLQPEDFATYYCQQHNEYPWTFGGGTKLEIK

SEQ ID NO: 140 - protein, 107 aa, Artificial
  7103-07 huVL4 Full-length sequence
DVQITQSPSSVSASVGETITINCRASKSISKYLAWYQQKPGKAPKLLIYSGSRLQSGVPSRFSGSGSGTDFTLTISSLQPEDFATYYCQQHNEYPWTFGGGTKLEIK

SEQ ID NO: 141 - protein, 107 aa, Artificial
  7103-07 huVL5 Full-length sequence
DIQMTQSPSSVSASVGETITITCRASKSISKYLAWYQQKPGKAPKLLIYSGSRLQSGVPSRFSGSGSGTDFTLTISSLQPEDFATYYCQQHNEYPWTFGGGTKLEIK

SEQ ID NO: 142 - protein, 17 aa, Artificial
  7103-01 huVH3 CDR2
GVNPSNGNTNFNENFKG

SEQ ID NO: 143 - protein, 17 aa, Artificial
  7103-07 huVH3 CDR2
EISSGGSHTFYADTVTG